European Patent Specification EP 4 525 938 B1, published March 11, 2026. Title: RADIOPHARMACEUTICAL COMPLEXES AND COMBINATIONS. Applicant: Bayer AG. The sequence listing filed with the application follows.

SEQUENCE LISTING (26 sequences)

SEQ ID NO: 1 - DNA, 1362 bp, unidentified
  source 1..1362: mol_type = genomic DNA
caggtgcagctcgtggaatcgggggggggcgtggtccagccggggcggtcgctccgcctctcgtgcgcagcctcgggcttcgccttcagccgctacggcatgcactgggtccgccaggcgcccggcaagggcctggagtgggtcgcggtcatctggtacgacgggtccaacaagtattatgcagactccgtcaagggtcggttcaccatcagccgggacaactccaagaacacccagtacctgcagatgaacagccttcgagcggaggacaccgcggtctactactgcgcccggggcggggatttcctgtactactactactatggcatggacgtctggggccagggtaccaccgtgaccgtatcctccgcatccactaagggcccgtccgttttcccgctggcaccttcgtcgaagagcacgtccgggggcacagccgcgctgggctgcctcgtgaaggactactttccggagcccgtcaccgtgtcatggaactcgggcgcgctcacgtccggcgtccacacgttcccggccgtattgcagagctcgggactctactccctgagctcggtcgtcaccgtgccctcctcgagcctcggcacccagacctacatctgcaacgtgaaccacaaaccctccaatacgaaggtggacaagcgcgtcgaaccgaagtcgtgcgacaagacccacacgtgcccgccgtgcccggcaccggagctgctcggcgggccctcggtcttcctgttcccgccgaagcccaaggacaccctgatgatctcgcgcaccccggaggtcacatgcgtggtcgtggacgtgtcccacgaagacccggaggtcaagttcaactggtacgtcgacggcgtcgaggtccacaacgcgaagaccaagccgcgggaggagcagtacaacagcacgtaccgcgtcgtttccgtcctcaccgtcttgcaccaggactggctgaacggcaaggagtacaagtgtaaggtgtccaacaaggccttgcccgcccccattgagaagaccatcagcaaggccaagggccagccccgcgagccgcaggtctacaccctgcccccgtcgcgcgaagaaatgacgaagaaccaggtctccctgacctgcctcgtcaaggggttctacccgtcggacatcgcagtggagtgggagtcgaacggccagcccgagaataactacaagacgacccccccagtcctggactccgacggcagcttcttcctttactccaagctgaccgtcgacaagtcgcggtggcagcagggcaacgtcttctcgtgctcggtgatgcacgaggcgctgcacaaccactacacccagaagtccctctcgctgtcgccgggcaagtga

SEQ ID NO: 2 - DNA, 645 bp, unidentified
  source 1..645: mol_type = genomic DNA
gacatccagatgacccagagccccagctccctgtccgcgtcggtcggagaccgggtcaccatcacctgccgcgcgtcgcagggcatctcgaactacctggcgtggtaccagcagaagaccggcaaggtgccgaagttccttatctacgaggcctctacgctccagtcgggagtcccgtcgcggttcagcgggggtggctccgggaccgacttcacgctgaccatctcgagtctccagccggaggacgtcgcgacctattactgtcagaactacaactcggcccccttcaccttcggcccgggcaccaaggtcgacatcaagcgcaccgtcgcggcgccgtccgtcttcatcttccccccgtcggacgagcagctcaagtccggcaccgcctcggtcgtgtgcctgctcaacaacttctacccccgagaggcaaaggtgcagtggaaggtcgacaacgccctgcagtccggcaactcgcaggagagcgtcacggagcaggacagcaaggacagtacctacagcctctcctccaccctgaccctgagtaaagccgactacgagaagcacaaggtgtacgcgtgcgaagtcacccaccagggcctctcgtcccccgtgaccaagtccttcaaccggggcgagtgctga

SEQ ID NO: 3 - protein, 453 aa, unidentified
QVQLVESGGGVVQPGRSLRLSCAASGFAFSRYGMHWVRQAPGKGLEWVAVIWYDGSNKYYADSVKGRFTISRDNSKNTQYLQMNSLRAEDTAVYYCARGGDFLYYYYYGMDVWGQGTTVTVSSASTKGPSVFPLAPSSKSTSGGTAALGCLVKDYFPEPVTVSWNSGALTSGVHTFPAVLQSSGLYSLSSVVTVPSSSLGTQTYICNVNHKPSNTKVDKRVEPKSCDKTHTCPPCPAPELLGGPSVFLFPPKPKDTLMISRTPEVTCVVVDVSHEDPEVKFNWYVDGVEVHNAKTKPREEQYNSTYRVVSVLTVLHQDWLNGKEYKCKVSNKALPAPIEKTISKAKGQPREPQVYTLPPSREEMTKNQVSLTCLVKGFYPSDIAVEWESNGQPENNYKTTPPVLDSDGSFFLYSKLTVDKSRWQQGNVFSCSVMHEALHNHYTQKSLSLSPGK

SEQ ID NO: 4 - protein, 214 aa, unidentified
DIQMTQSPSSLSASVGDRVTITCRASQGISNYLAWYQQKTGKVPKFLIYEASTLQSGVPSRFSGGGSGTDFTLTISSLQPEDVATYYCQNYNSAPFTFGPGTKVDIKRTVAAPSVFIFPPSDEQLKSGTASVVCLLNNFYPREAKVQWKVDNALQSGNSQESVTEQDSKDSTYSLSSTLTLSKADYEKHKVYACEVTHQGLSSPVTKSFNRGEC

SEQ ID NO: 5 - protein, 5 aa, unidentified
RYGMH

SEQ ID NO: 6 - protein, 17 aa, unidentified
VIWYDGSNKYYADSVKG

SEQ ID NO: 7 - protein, 14 aa, unidentified
GGDFLYYYYYGMDV

SEQ ID NO: 8 - protein, 11 aa, unidentified
RASQGISNYLA

SEQ ID NO: 9 - protein, 7 aa, unidentified
EASTLQS

SEQ ID NO: 10 - protein, 9 aa, unidentified
QNYNSAPFT

SEQ ID NO: 11 - protein, 444 aa, unidentified
EVQLVQSGPEVKKPGATVKISCKTSGYTFTEYTIHWVKQAPGKGLEWIGNINPNNGGTTYNQKFEDKATLTVDKSTDTAYMELSSLRSEDTAVYYCAAGWNFDYWGQGTLLTVSSASTKGPSVFPLAPSSKSTSGGTAALGCLVKDYFPEPVTVSWNSGALTSGVHTFPAVLQSSGLYSLSSVVTVPSSSLGTQTYICNVNHKPSNTKVDKKVEPKSCDKTHTCPPCPAPELLGGPSVFLFPPKPKDTLMISRTPEVTCVVVDVSHEDPEVKFNWYVDGVEVHNAKTKPREEQYNSTYRVVSVLTVLHQDWLNGKEYKCKVSNKALPAPIEKTISKAKGQPREPQVYTLPPSRDELTKNQVSLTCLVKGFYPSDIAVEWESNGQPENNYKTTPPVLDSDGSFFLYSKLTVDKSRWQQGNVFSCSVMHEALHNHYTQKSLSLSPG

SEQ ID NO: 12 - protein, 214 aa, unidentified
DIQMTQSPSSLSTSVGDRVTLTCKASQDVGTAVDWYQQKPGPSPKLLIYWASTRHTGIPSRFSGSGSGTDFTLTISSLQPEDFADYYCQQYNSYPLTFGPGTKVDIKRTVAAPSVFIFPPSDEQLKSGTASVVCLLNNFYPREAKVQWKVDNALQSGNSQESVTEQDSKDSTYSLSSTLTLSKADYEKHKVYACEVTHQGLSSPVTKSFNRGEC

SEQ ID NO: 13 - protein, 4 aa, unidentified
YTIH

SEQ ID NO: 14 - protein, 17 aa, unidentified
NINPNNGGTTYNQKFED

SEQ ID NO: 15 - protein, 6 aa, unidentified
GWNFDY

SEQ ID NO: 16 - protein, 11 aa, unidentified
KASQDVGTAVD

SEQ ID NO: 17 - protein, 7 aa, unidentified
WASTRHT

SEQ ID NO: 18 - protein, 9 aa, unidentified
QQYNSYPLT

SEQ ID NO: 19 - protein, 445 aa, unidentified
EVQLVQSGAEVKKPGASVKVSCKASGYTFTEYTIHWVRQAPGKGLEWIGNINPNNGGTTYNQKFEDRVTITVDKSTSTAYMELSSLRSEDTAVYYCAAGWNFDYWGQGTTVTVSSASTKGPSVFPLAPSSKSTSGGTAALGCLVKDYFPEPVTVSWNSGALTSGVHTFPAVLQSSGLYSLSSVVTVPSSSLGTQTYICNVNHKPSNTKVDKRVEPKSCDKTHTCPPCPAPELLGGPSVFLFPPKPKDTLMISRTPEVTCVVVDVSHEDPEVKFNWYVDGVEVHNAKTKPREEQYNSTYRVVSVLTVLAQDWLNGKEYKCKVSNKALPAPIEKTISKAKGQPREPQVYTLPPSREEMTKNQVSLTCLVKGFYPSDIAVEWESNGQPENNYKTTPPVLDSDGSFFLYSKLTVDKSRWQQGNVFSCSVMHEALHNQYTQKSLSLSPGK

SEQ ID NO: 20 - protein, 214 aa, unidentified
DIQMTQSPSTLSASVGDRVTITCKASQDVGTAVDWYQQKPGQAPKLLIYWASTRHTGVPDRFSGSGSGTDFTLTISRLQPEDFAVYYCQQYNSYPLTFGQGTKVDIKRTVAAPSVFIFPPSDEQLKSGTASVVCLLNNFYPREAKVQWKVDNALQSGNSQESVTEQDSKDSTYSLSSTLTLSKADYEKHKVYACEVTHQGLSSPVTKSFNRGEC

SEQ ID NO: 21 - protein, 5 aa, unidentified
EYTIH

SEQ ID NO: 22 - protein, 17 aa, unidentified
NINPNNGGTTYNQKFED

SEQ ID NO: 23 - protein, 6 aa, unidentified
GWNFDY

SEQ ID NO: 24 - protein, 11 aa, unidentified
KASQDVGTAVD

SEQ ID NO: 25 - protein, 7 aa, unidentified
WASTRHT

SEQ ID NO: 26 - protein, 9 aa, unidentified
QQYNSYPLT